European Patent Application EP 4 177 348 A1, published May 10, 2023. Title: VACCINES AGAINST HEPATITIS B VIRUS. Applicant: Hookipa Biotech GmbH. The sequence listing filed with the application follows.

SEQUENCE LISTING (26 sequences)

SEQ ID NO: 1 - DNA, 846 bp, synthetic construct
  source 1..846: mol_type = other DNA; note = HBV pre-S2/S ORF
atgcagtggaattccacaaccttccaccaaactctgcaagatcccagagtgagaggcctgtatttccctgctggtggctccagttcaggaacagtcaaccctgttctgaccactgcctctcccttgtcatcaatcttctccaggattggggaccctgctctgaacatggagaacatcacatcaggattcctgggaccccttcttgtgttgcaggcagggtttttcttgttgacaagaatcctcacaatccctcagagtctggactcttggtggacttctctcaattttctggggggaaccacagtgtgtcttggccaaaattctcagtccccaacctccaatcactcaccaacctcttgtcctccaacttgtcctggttacagatggatgtgtctgaggagattcatcatcttcctcttcatcctgctgctgtgcctcatcttcttgttggttcttctggactatcaaggaatgttgccagtttgtcctctgattccaggatcctcaacaaccagcactggaccatgcaggacctgcatgaccactgctcaaggaacctcaatgtatccctcctgttgctgcaccaaaccttcagatggaaattgcacctgcattcccatcccatcatcctgggcttttggaaaattcctttgggagtgggcctcagccagattctcctggctcagtttgctggtgccatttgttcagtggtttgttgggctttcccccactgtttggctttcagtgatttggatgatgtggtattgggggccaagtctgtacagcatcttgagtccctttttgcctctgttgccaattttcttttgtctttgggtctacatttaa

SEQ ID NO: 2 - DNA, 552 bp, synthetic construct
  source 1..552: mol_type = other DNA; note = HBV HBc ORF
atggacattgacccttacaaagaatttggagcaactgtggagttgctctcctttttgccttctgacttctttccttcagtgagagatcttcttgacactgcctcagctctgtacagggaagccttggagtctcctgagcattgttcacctcaccacactgcactcaggcaagcaattctttgctggggggaactcatgactctggcaacctgggtgggtgtcaatttggaagatccagcctcaagagaccttgtggtcagttatgtcaacacaaacatgggcctgaagttcaggcaactcttgtggtttcacatttcttgtctcacttttggaagagaaacagtcattgagtatttggtgtcttttggagtgtggatcaggactcctccagcttacagaccaccaaatgccccaatcctgtcaacacttccagagaccactgttgtcagaagaagaggcaggtcccccagaagaagaactccctcaccaagaagaagaaggtctcaatctcccagaaggagaagatctcaatcaagggaatctcaatgttag

SEQ ID NO: 3 - DNA, 1719 bp, synthetic construct
  source 1..1719: mol_type = other DNA; note = HBV HBs-HBc fusion protein ORF
atggggcagaatctttccaccagcaatcctctgggattctttccagaccaccagttggatccagccttcagagcaaacactgcaaatccagattgggacttcaatcccaacaaggacacctggccagatgccaacaaggtgggagctggagcatttgggctgggtttcaccccaccccatggaggccttttggggtggagccctcaggctcagggcattctgcaaactttgccagcaaatccacctcctgcctccaccaacaggcagtcaggaaggcagcccacccctctgtctccacctttgagaaacactcatcctcaggccatgcagtggaattccacaaccttccaccaaactctgcaagatcccagagtgagaggcctgtatttccctgctggtggctccagttcaggaacagtcaaccctgttctgaccactgcctctcccttgtcatcaatcttctccaggattggggaccctgctctgaacatggagaacatcacatcaggattcctgggaccccttcttgtgttgcaggcagggtttttcttgttgacaagaatcctcacaatccctcagagtctggactcttggtggacttctctcaattttctggggggaaccacagtgtgtcttggccaaaattctcagtccccaacctccaatcactcaccaacctcttgtcctccaacttgtcctggttacagatggatgtgtctgaggagattcatcatcttcctcttcatcctgctgctgtgcctcatcttcttgttggttcttctggactatcaaggaatgttgccagtttgtcctctgattccaggatcctcaacaaccagcactggaccatgcaggacctgcatgaccactgctcaaggaacctcaatgtatccctcctgttgctgcaccaaaccttcagatggaaattgcacctgcattcccatcccatcatcctgggcttttggaaaattcctttgggagtgggcctcagccagattctcctggctcagtttgctggtgccatttgttcagtggtttgttgggctttcccccactgtttggctttcagtgatttggatgatgtggtattgggggccaagtctgtacagcatcttgagtccctttttgcctctgttgccaattttcttttgtctttgggtctacattatggacattgacccttacaaagaatttggagcaactgtggagttgctctcctttttgccttctgacttctttccttcagtgagagatcttcttgacactgcctcagctctgtacagggaagccttggagtctcctgagcattgttcacctcaccacactgcactcaggcaagcaattctttgctggggggaactcatgactctggcaacctgggtgggtgtcaatttggaagatccagcctcaagagaccttgtggtcagttatgtcaacacaaacatgggcctgaagttcaggcaactcttgtggtttcacatttcttgtctcacttttggaagagaaacagtcattgagtatttggtgtcttttggagtgtggatcaggactcctccagcttacagaccaccaaatgccccaatcctgtcaacacttccagagaccactgttgtcagaagaagaggcaggtcccccagaagaagaactccctcaccaagaagaagaaggtctcaatctcccagaaggagaagatctcaatcaagggaatctcaatgttag

SEQ ID NO: 4 - DNA, 3599 bp, synthetic construct
  source 1..3599: mol_type = other DNA; note = cDNA of LCMV S segment expressing HBV HBs-HBc fusion protein
gcgcaccggggatcctaggctttttggattgcgctttcctctagatcaactgggtgtcaggccctatcctacagaaggatggggcagaatctttccaccagcaatcctctgggattctttccagaccaccagttggatccagccttcagagcaaacactgcaaatccagattgggacttcaatcccaacaaggacacctggccagatgccaacaaggtgggagctggagcatttgggctgggtttcaccccaccccatggaggccttttggggtggagccctcaggctcagggcattctgcaaactttgccagcaaatccacctcctgcctccaccaacaggcagtcaggaaggcagcccacccctctgtctccacctttgagaaacactcatcctcaggccatgcagtggaattccacaaccttccaccaaactctgcaagatcccagagtgagaggcctgtatttccctgctggtggctccagttcaggaacagtcaaccctgttctgaccactgcctctcccttgtcatcaatcttctccaggattggggaccctgctctgaacatggagaacatcacatcaggattcctgggaccccttcttgtgttgcaggcagggtttttcttgttgacaagaatcctcacaatccctcagagtctggactcttggtggacttctctcaattttctggggggaaccacagtgtgtcttggccaaaattctcagtccccaacctccaatcactcaccaacctcttgtcctccaacttgtcctggttacagatggatgtgtctgaggagattcatcatcttcctcttcatcctgctgctgtgcctcatcttcttgttggttcttctggactatcaaggaatgttgccagtttgtcctctgattccaggatcctcaacaaccagcactggaccatgcaggacctgcatgaccactgctcaaggaacctcaatgtatccctcctgttgctgcaccaaaccttcagatggaaattgcacctgcattcccatcccatcatcctgggcttttggaaaattcctttgggagtgggcctcagccagattctcctggctcagtttgctggtgccatttgttcagtggtttgttgggctttcccccactgtttggctttcagtgatttggatgatgtggtattgggggccaagtctgtacagcatcttgagtccctttttgcctctgttgccaattttcttttgtctttgggtctacattatggacattgacccttacaaagaatttggagcaactgtggagttgctctcctttttgccttctgacttctttccttcagtgagagatcttcttgacactgcctcagctctgtacagggaagccttggagtctcctgagcattgttcacctcaccacactgcactcaggcaagcaattctttgctggggggaactcatgactctggcaacctgggtgggtgtcaatttggaagatccagcctcaagagaccttgtggtcagttatgtcaacacaaacatgggcctgaagttcaggcaactcttgtggtttcacatttcttgtctcacttttggaagagaaacagtcattgagtatttggtgtcttttggagtgtggatcaggactcctccagcttacagaccaccaaatgccccaatcctgtcaacacttccagagaccactgttgtcagaagaagaggcaggtcccccagaagaagaactccctcaccaagaagaagaaggtctcaatctcccagaaggagaagatctcaatcaagggaatctcaatgttagagaacagcgcctccctgactctccacctcgaaagaggtggagagtcagggaggcccagagggtcttagagtgtcacaacatttgggcctctaaaaattaggtcatgtggcagaatgttgtgaacagttttcagatctgggagccttgctttggaggcgctttcaaaaatgatgcagtccatgagtgcacagtgcggggtgatctctttcttctttttgtcccttactattccagtatgcatcttacacaaccagccatatttgtcccacactttatcttcatactccctcgaagcttccctggtcatttcaacatcgataagcttaatgtccttcctattttgtgagtccagaagctttctgatgtcatcggagccttgacagcttagaaccatcccctgcggaagagcacctataactgacgaggtcaacccgggttgcgcattgaagaggtcggcaagatccatgccgtgtgagtacttggaatcttgcttgaattgtttttgatcaacgggttccctgtaaaagtgtatgaactgcccgttctgtggttggaaaattgctatttccactggatcattaaatctaccctcaatgtcaatccatgtaggagcgttggggtcaattcctcccatgaggtcttttaaaagcattgtctggctgtagcttaagcccacctgaggtggacctgctgctccaggcgctggcctgggtgagttgactgcaggtttctcgcttgtgagatcaattgttgtgttttcccatgctctccccacaatcgatgttctacaagctatgtatggccatccttcacctgaaaggcaaactttatagaggatgttttcataagggttcctgtccccaacttggtctgaaacaaacatgttgagttttctcttggccccgagaactgccttcaagagatcctcgctgttgcttggcttgatcaaaattgactctaacatgttacccccatccaacagggctgcccctgccttcacggcagcaccaagactaaagttatagccagaaatgttgatgctggactgctgttcagtgatgacccccagaactgggtgcttgtctttcagcctttcaagatcattaagatttggatacttgactgtgtaaagcaagccaaggtctgtgagcgcttgtacaacgtcattgagcggagtctgtgactgtttggccatacaagccatagttagacttggcattgtgccaaattgattgttcaaaagtgatgagtctttcacatcccaaactcttaccacaccacttgcaccctgctgaggctttctcatcccaactatctgtaggatctgagatctttggtctagttgctgtgttgttaagttccccatatatacccctgaagcctggggcctttcagacctcatgatcttggccttcagcttctcaaggtcagccgcaagagacatcagttcttctgcactgagcctccccactttcaaaacattcttctttgatgttgactttaaatccacaagagaatgtacagtctggttgagacttctgagtctctgtaggtctttgtcatctctcttttccttcctcatgatcctctgaacattgctgacctcagagaagtccaacccattcagaaggttggttgcatccttaatgacagcagccttcacatctgatgtgaagctctgcaattctcttctcaatgcttgcgtccattggaagctcttaacttccttagacaaggacatcttgttgctcaatggtttctcaagacaaatgcgcaatcaaatgcctaggatccactgtgcg

SEQ ID NO: 5 - DNA, 2432 bp, synthetic construct
  source 1..2432: mol_type = other DNA; note = cDNA of LCMV S segment expressing the HBc ORF
gcgcaccggggatcctaggctttttggattgcgctttcctctagatcaactgggtgtcaggccctatcctacagaaggatggacattgacccttacaaagaatttggagcaactgtggagttgctctcctttttgccttctgacttctttccttcagtgagagatcttcttgacactgcctcagctctgtacagggaagccttggagtctcctgagcattgttcacctcaccacactgcactcaggcaagcaattctttgctggggggaactcatgactctggcaacctgggtgggtgtcaatttggaagatccagcctcaagagaccttgtggtcagttatgtcaacacaaacatgggcctgaagttcaggcaactcttgtggtttcacatttcttgtctcacttttggaagagaaacagtcattgagtatttggtgtcttttggagtgtggatcaggactcctccagcttacagaccaccaaatgccccaatcctgtcaacacttccagagaccactgttgtcagaagaagaggcaggtcccccagaagaagaactccctcaccaagaagaagaaggtctcaatctcccagaaggagaagatctcaatcaagggaatctcaatgttagagaacagcgcctccctgactctccacctcgaaagaggtggagagtcagggaggcccagagggtcttagagtgtcacaacatttgggcctctaaaaattaggtcatgtggcagaatgttgtgaacagttttcagatctgggagccttgctttggaggcgctttcaaaaatgatgcagtccatgagtgcacagtgcggggtgatctctttcttctttttgtcccttactattccagtatgcatcttacacaaccagccatatttgtcccacactttatcttcatactccctcgaagcttccctggtcatttcaacatcgataagcttaatgtccttcctattttgtgagtccagaagctttctgatgtcatcggagccttgacagcttagaaccatcccctgcggaagagcacctataactgacgaggtcaacccgggttgcgcattgaagaggtcggcaagatccatgccgtgtgagtacttggaatcttgcttgaattgtttttgatcaacgggttccctgtaaaagtgtatgaactgcccgttctgtggttggaaaattgctatttccactggatcattaaatctaccctcaatgtcaatccatgtaggagcgttggggtcaattcctcccatgaggtcttttaaaagcattgtctggctgtagcttaagcccacctgaggtggacctgctgctccaggcgctggcctgggtgagttgactgcaggtttctcgcttgtgagatcaattgttgtgttttcccatgctctccccacaatcgatgttctacaagctatgtatggccatccttcacctgaaaggcaaactttatagaggatgttttcataagggttcctgtccccaacttggtctgaaacaaacatgttgagttttctcttggccccgagaactgccttcaagagatcctcgctgttgcttggcttgatcaaaattgactctaacatgttacccccatccaacagggctgcccctgccttcacggcagcaccaagactaaagttatagccagaaatgttgatgctggactgctgttcagtgatgacccccagaactgggtgcttgtctttcagcctttcaagatcattaagatttggatacttgactgtgtaaagcaagccaaggtctgtgagcgcttgtacaacgtcattgagcggagtctgtgactgtttggccatacaagccatagttagacttggcattgtgccaaattgattgttcaaaagtgatgagtctttcacatcccaaactcttaccacaccacttgcaccctgctgaggctttctcatcccaactatctgtaggatctgagatctttggtctagttgctgtgttgttaagttccccatatatacccctgaagcctggggcctttcagacctcatgatcttggccttcagcttctcaaggtcagccgcaagagacatcagttcttctgcactgagcctccccactttcaaaacattcttctttgatgttgactttaaatccacaagagaatgtacagtctggttgagacttctgagtctctgtaggtctttgtcatctctcttttccttcctcatgatcctctgaacattgctgacctcagagaagtccaacccattcagaaggttggttgcatccttaatgacagcagccttcacatctgatgtgaagctctgcaattctcttctcaatgcttgcgtccattggaagctcttaacttccttagacaaggacatcttgttgctcaatggtttctcaagacaaatgcgcaatcaaatgcctaggatccactgtgcg

SEQ ID NO: 6 - DNA, 2726 bp, synthetic construct
  source 1..2726: mol_type = other DNA; note = cDNA of LCMV S segment expressing the pre-S2/S ORF
gcgcaccggggatcctaggctttttggattgcgctttcctctagatcaactgggtgtcaggccctatcctacagaaggatgcagtggaattccacaaccttccaccaaactctgcaagatcccagagtgagaggcctgtatttccctgctggtggctccagttcaggaacagtcaaccctgttctgaccactgcctctcccttgtcatcaatcttctccaggattggggaccctgctctgaacatggagaacatcacatcaggattcctgggaccccttcttgtgttgcaggcagggtttttcttgttgacaagaatcctcacaatccctcagagtctggactcttggtggacttctctcaattttctggggggaaccacagtgtgtcttggccaaaattctcagtccccaacctccaatcactcaccaacctcttgtcctccaacttgtcctggttacagatggatgtgtctgaggagattcatcatcttcctcttcatcctgctgctgtgcctcatcttcttgttggttcttctggactatcaaggaatgttgccagtttgtcctctgattccaggatcctcaacaaccagcactggaccatgcaggacctgcatgaccactgctcaaggaacctcaatgtatccctcctgttgctgcaccaaaccttcagatggaaattgcacctgcattcccatcccatcatcctgggcttttggaaaattcctttgggagtgggcctcagccagattctcctggctcagtttgctggtgccatttgttcagtggtttgttgggctttcccccactgtttggctttcagtgatttggatgatgtggtattgggggccaagtctgtacagcatcttgagtccctttttgcctctgttgccaattttcttttgtctttgggtctacatttaaagaacagcgcctccctgactctccacctcgaaagaggtggagagtcagggaggcccagagggtcttagagtgtcacaacatttgggcctctaaaaattaggtcatgtggcagaatgttgtgaacagttttcagatctgggagccttgctttggaggcgctttcaaaaatgatgcagtccatgagtgcacagtgcggggtgatctctttcttctttttgtcccttactattccagtatgcatcttacacaaccagccatatttgtcccacactttatcttcatactccctcgaagcttccctggtcatttcaacatcgataagcttaatgtccttcctattttgtgagtccagaagctttctgatgtcatcggagccttgacagcttagaaccatcccctgcggaagagcacctataactgacgaggtcaacccgggttgcgcattgaagaggtcggcaagatccatgccgtgtgagtacttggaatcttgcttgaattgtttttgatcaacgggttccctgtaaaagtgtatgaactgcccgttctgtggttggaaaattgctatttccactggatcattaaatctaccctcaatgtcaatccatgtaggagcgttggggtcaattcctcccatgaggtcttttaaaagcattgtctggctgtagcttaagcccacctgaggtggacctgctgctccaggcgctggcctgggtgagttgactgcaggtttctcgcttgtgagatcaattgttgtgttttcccatgctctccccacaatcgatgttctacaagctatgtatggccatccttcacctgaaaggcaaactttatagaggatgttttcataagggttcctgtccccaacttggtctgaaacaaacatgttgagttttctcttggccccgagaactgccttcaagagatcctcgctgttgcttggcttgatcaaaattgactctaacatgttacccccatccaacagggctgcccctgccttcacggcagcaccaagactaaagttatagccagaaatgttgatgctggactgctgttcagtgatgacccccagaactgggtgcttgtctttcagcctttcaagatcattaagatttggatacttgactgtgtaaagcaagccaaggtctgtgagcgcttgtacaacgtcattgagcggagtctgtgactgtttggccatacaagccatagttagacttggcattgtgccaaattgattgttcaaaagtgatgagtctttcacatcccaaactcttaccacaccacttgcaccctgctgaggctttctcatcccaactatctgtaggatctgagatctttggtctagttgctgtgttgttaagttccccatatatacccctgaagcctggggcctttcagacctcatgatcttggccttcagcttctcaaggtcagccgcaagagacatcagttcttctgcactgagcctccccactttcaaaacattcttctttgatgttgactttaaatccacaagagaatgtacagtctggttgagacttctgagtctctgtaggtctttgtcatctctcttttccttcctcatgatcctctgaacattgctgacctcagagaagtccaacccattcagaaggttggttgcatccttaatgacagcagccttcacatctgatgtgaagctctgcaattctcttctcaatgcttgcgtccattggaagctcttaacttccttagacaaggacatcttgttgctcaatggtttctcaagacaaatgcgcaatcaaatgcctaggatccactgtgcg

SEQ ID NO: 7 - DNA, 7229 bp, synthetic construct
  source 1..7229: mol_type = other DNA; note = lymphocytic choriomeningitis virus clone 13 segment L (GenBank: DQ361066.1)
gcgcaccggggatcctaggcgtttagttgcgctgtttggttgcacaactttcttcgtgaggctgtcagaagtggacctggctgatagcgatgggtcaaggcaagtccagagaggagaaaggcaccaatagtacaaacagggccgaaatcctaccagataccacctatcttggccctttaagctgcaaatcttgctggcagaaatttgacagcttggtaagatgccatgaccactacctttgcaggcactgtttaaaccttctgctgtcagtatccgacaggtgtcctctttgtaaatatccattaccaaccagattgaagatatcaacagccccaagctctccacctccctacgaagagtaacaccgtccggccccggccccgacaaacagcccagcacaagggaaccgcacgtcacccaacgcacacagacacagcacccaacacagaacacgcacacacacacacacacacacccacacgcacgcgcccccaccaccggggggcgcccccccccggggggcggccccccgggagcccgggcggagccccacggagatgcccatcagtcgatgtcctcggccaccgacccgcccagccaatcgtcgcaggacctccccttgagtctaaacctgccccccactgtttcatacatcaaagtgctcctagatttgctaaaacaaagtctgcaatccttaaaggcgaaccagtctggcaaaagcgacagtggaatcagcagaatagatctgtctatacatagttcctggaggattacacttatctctgaacccaacaaatgttcaccagttctgaatcgatgcaggaagaggttcccaaggacatcactaatcttttcatagccctcaagtcctgctagaaagactttcatgtccttggtctccagcttcacaatgatattttggacaaggtttcttccttcaaaaagggcacccatctttacagtcagtggcacaggctcccactcaggtccaactctctcaaagtcaatagatctaatcccatccagtattcttttggagcccaacaactcaagctcaagagaatcaccaagtatcaagggatcttccatgtaatcctcaaactcttcagatctgatatcaaagacaccatcgttcaccttgaagacagagtctgtcctcagtaagtggaggcattcatccaacattcttctatctatctcacccttaaagaggtgagagcatgataaaagttcagccacacctggattctgtaattggcacctaaccaagaatatcaatgaaaatttccttaaacagtcagtattattctgattgtgcgtaaagtccactgaaattgaaaactccaataccccttttgtgtagttgagcatgtagtcccacagatcctttaaggatttaaatgcctttgggtttgtcaggccctgcctaatcaacatggcagcattacacacaacatctcccattcggtaagagaaccacccaaaaccaaactgcaaatcattcctaaacataggcctctccacatttttgttcaccacctttgagacaaatgattgaaaggggcccagtgcctcagcaccatcttcagatggcatcatttctttatgagggaaccatgaaaaattgcctaatgtcctggttgttgcaacaaattctcgaacaaatgattcaaaatacacctgttttaagaagttcttgcagacatccctcgtgctaacaacaaattcatcaaccagactggagtcagatcgctgatgagaattggcaaggtcagaaaacagaacagtgtaatgttcatcccttttccacttaacaacatgagaaatgagtgacaaggattctgagttaatatcaattaaaacacagaggtcaaggaatttaattctgggactccacctcatgttttttgagctcatgtcagacataaatggaagaagctgatcctcaaagatcttgggatatagccgcctcacagattgaatcacttggttcaaattcactttgtcctccagtagccttgagctctcaggctttcttgctacataatcacatgggtttaagtgcttaagagttaggttctcactgttattcttccctttggtcggttctgctaggacccaaacacccaactcaaaagagttgctcaatgaaatacaaatgtagtcccaaagaagaggccttaaaaggcatatatgatcacggtgggcttctggatgagactgtttgtcacaaatgtacagcgttataccatcccgattgcaaactcttgtcacatgatcatctgtggttagatcctcaagcagctttttgatatacagattttccctatttttgtttctcacacacctgcttcctagagttttgcaaaggcctataaagccagatgagatacaactctggaaagctgacttgttgattgcttctgacagcagcttctgtgcaccccttgtgaatttactacaaagtttgttctggagtgtcttgatcaatgatgggattctttcctcttggaaagtcatcactgatggataaaccaccttttgtcttaaaaccatccttaatgggaacatttcattcaaattcaaccagttaacatctgctaactgattcagatcttcttcaagaccgaggaggtctcccaattgaagaatggcctcctttttatctctgttaaataggtctaagaaaaattcttcattaaattcaccatttttgagcttatgatgcagtttccttacaagctttcttacaacctttgtttcattaggacacagttcctcaatgagtctttgtattctgtaacctctagaaccatccagccaatctttcacatcagtgttggtattcagtagaaatggatccaaagggaaattggcatactttaggaggtccagtgttctcctttggatactattaactagggagactgggacgccatttgcgatggcttgatctgcaattgtatctattgtttcacaaagttgatgtggctctttacacttgacattgtgtagcgctgcagatacaaactttgtgagaagagggacttcctccccccatacatagaatctagatttaaattctgcagcgaacctcccagccacactttttgggctgataaatttgtttaacaagccgctcagatgagattggaattccaacaggacaaggacttcctccggatcacttacaaccaggtcactcagcctcctatcaaataaagtgatctgatcatcacttgatgtgtaagcctctggtctttcgccaaagataacaccaatgcagtagttgatgaacctctcgctaagcaaaccatagaagtcagaagcattatgcaagattccctgccccatatcaataaggctggatatatgggatggcactatccccatttcaaaatattgtctgaaaattctctcagtaacagttgtttctgaacccctgagaagttttagcttcgacttgacatatgatttcatcattgcattcacaacaggaaaggggacctcgacaagcttatgcatgtgccaagttaacaaagtgctaacatgatctttcccggaacgcacatactggtcatcacctagtttgagattttgtagaaacattaagaacaaaaatgggcacatcattggtccccatttgctgtgatccatactatagtttaagaacccttcccgcacattgatagtcattgacaagattgcattttcaaattccttatcattgtttaaacaggagcctgaaaagaaacttgaaaaagactcaaaataatcttctattaaccttgtgaacatttttgtcctcaaatctccaatatagagttctctatttcccccaacctgctctttataagatagtgcaaatttcagccttccagagtcaggacctactgaggtgtatgatgttggtgattcttctgagtagaagcacagatttttcaaagcagcactcatacattgtgtcaacgacagagctttactaagggactcagaattactttccctctcactgattctcacgtcttcttccagtttgtcccagtcaaatttgaaattcaagccttgcctttgcatatgcctgtatttccctgagtacgcatttgcattcatttgcaacagaatcatcttcatgcaagaaaaccaatcattctcagaaaagaactttctacaaaggttttttgccatctcatcgaggccacactgatctttaatgactgaggtgaaatacaaaggtgacagctctgtggaaccctcaacagcctcacagataaatttcatgtcatcattggttagacatgatgggtcaaagtcttctactaaatggaaagatatttctgacaagataacttttcttaagtgagccatcttccctgttagaataagctgtaaatgatgtagtccttttgtatttgtaagtttttctccatctcctttgtcattggccctcctacctcttctgtaccgtgctattgtggtgttgaccttttcttcgagacttttgaagaagcttgtctcttcttctccatcaaaacatatttctgccaggttgtcttccgatctccctgtctcttctcccttggaaccgatgaccaatctagagactaacttggaaactttatattcatagtctgagtggctcaacttatacttttgttttcttacgaaactctccgtaatttgactcacagcactaacaagcaatttgttaaagtcatattccagaagtcgttctccatttagatgcttattaaccaccacacttttgttactagcaagatctaatgctgtcgcacatccagagttagtcatgggatctaggctgtttagcttcttctctcctttgaaaattaaagtgccgttgttaaatgaagacaccattaggctaaaggcttccagattaacacctggagttgtatgctgacagtcaatttctttactagtgaatctcttcatttgctcatagaacacacattcttcctcaggagtgattgcttccttggggttgacaaaaaaaccaaattgacttttgggctcaaagaacttttcaaaacattttatctgatctgttagcctgtcaggggtctcctttgtgatcaaatgacacaggtatgacacattcaacataaatttaaattttgcactcaacaacaccttctcaccagtaccaaaaatagtttttattaggaatctaagcagcttatacaccaccttctcagcaggtgtgatcagatcctccctcaacttatccattaatgatgtagatgaaaaatctgacactattgccatcaccaaatatctgacactctgtacctgcttttgatttctctttgttgggttggtgagcattagcaacaatagggtcctcagtgcaacctcaatgtcggtgagacagtctttcaaatcaggacatgatctaatccatgaaatcatgatgtctatcatattgtataagacctcatctgaaaaaattggtaaaaagaaccttttaggatctgcatagaaggaaattaaatgaccatccgggccttgtatggagtagcaccttgaagattctccagtcttctggtataataggtggtattcttcagagtccagttttattacttggcaaaacacttctttgcattctaccacttgatatctcacagaccctatttgattttgccttagtctagcaactgagctagttttcatactgtttgttaaggccagacaaacagatgataatcttctcaggctctgtatgttcttcagctgctctgtgctgggttggaaattgtaatcttcaaacttcgtataatacattatcgggtgagctccaattttcataaagttctcaaattcagtgaatggtatgtggcattcttgctcaaggtgttcagacagtccgtaatgctcgaaactcagtcccaccactaacaggcatttttgaatttttgcaatgaactcactaatagatgccctaaacaattcctcaaaagacacctttctaaacacctttgacttttttctattcctcaaaagtctaatgaactcctctttagtgctgtgaaagcttaccagcctatcattcacactactatagcaacaacccacccagtgtttatcattttttaaccctttgaatttcgactgttttatcaatgaggaaagacacaaaacatccagatttaacaactgtctccttctagtattcaacagtttcaaactcttgactttgtttaacatagagaggagcctctcatattcagtgctagtctcacttcccctttcgtgcccatgggtctctgcagttatgaatctcatcaaaggacaggattcgactgcctccctgcttaatgttaagatatcatcactatcagcaaggttttcatagagctcagagaattccttgatcaagccttcagggtttactttctgaaagtttctctttaatttcccactttctaaatctcttctaaacctgctgaaaagagagtttattccaaaaaccacatcatcacagctcatgttggggttgatgccttcgtggcacatcctcataatttcatcattgtgagttgacctcgcatctttcagaattttcatagagtccataccggagcgcttgtcgatagtagtcttcagggactcacagagtctaaaatattcagactcttcaaagactttctcattttggttagaatactccaaaagtttgaataaaaggtctctaaatttgaagtttgcccactctggcataaaactattatcataatcacaacgaccatctactattggaactaatgtgacacccgcaacagcaaggtcttccctgatgcatgccaatttgttagtgtcctctataaatttcttctcaaaactggctggagtgctcctaacaaaacactcaagaagaatgagagaattgtctatcagcttgtaaccatcaggaatgataagtggtagtcctgggcatacaattccagactccaccaaaattgtttccacagacttatcgtcgtggttgtgtgtgcagccactcttgtctgcactgtctatttcaatgcagcgtgacagcaacttgagtccctcaatcagaaccattctgggttccctttgtcccagaaagttgagtttctgccttgacaacctctcatcctgttctatatagtttaaacataactctctcaattctgagatgatttcatccattgcgcatcaaaaagcctaggatcctcggtgcg

SEQ ID NO: 8 - protein, 8 aa, synthetic construct
  source 1..8: note = HBV HBs protein-derived epitope
VWLSVIWM

SEQ ID NO: 9 - protein, 12 aa, synthetic construct
  source 1..12: note = HBV HBs protein-derived epitope
IPQSLDSWWTSL

SEQ ID NO: 10 - protein, 8 aa, synthetic construct
  source 1..8: note = HBV HBc protein-derived epitope
MGLKFRQL

SEQ ID NO: 11 - DNA, 3376 bp, synthetic construct
  source 1..3376: mol_type = other DNA; note = lymphocytic choriomeningitis virus segment S, complete cDNA sequence
cgcaccggggatcctaggctttttggattgcgctttcctctagatcaactgggtgtcaggccctatcctacagaaggatgggtcagattgtgacaatgtttgaggctctgcctcacatcatcgatgaggtgatcaacattgtcattattgtgcttatcgtgatcacgggtatcaaggctgtctacaattttgccacctgtgggatattcgcattgatcagtttcctacttctggctggcaggtcctgtggcatgtacggtcttaagggacccgacatttacaaaggagtttaccaatttaagtcagtggagtttgatatgtcacatctgaacctgaccatgcccaacgcatgttcagccaacaactcccaccattacatcagtatggggacttctggactagaattgaccttcaccaatgattccatcatcagtcacaacttttgcaatctgacctctgccttcaacaaaaagacctttgaccacacactcatgagtatagtttcgagcctacacctcagtatcagagggaactccaactataaggcagtatcctgcgacttcaacaatggcataaccatccaatacaacttgacattctcagatcgacaaagtgctcagagccagtgtagaaccttcagaggtagagtcctagatatgtttagaactgccttcggggggaaatacatgaggagtggctggggctggacaggctcagatggcaagaccacctggtgtagccagacgagttaccaatacctgattatacaaaatagaacctgggaaaaccactgcacatatgcaggtccttttgggatgtccaggattctcctttcccaagagaagactaagttcttcactaggagactagcgggcacattcacctggactttgtcagactcttcaggggtggagaatccaggtggttattgcctgaccaaatggatgattcttgctgcagagcttaagtgtttcgggaacacagcagttgcgaaatgcaatgtaaatcatgatgccgaattctgtgacatgctgcgactaattgactacaacaaggctgctttgagtaagttcaaagaggacgtagaatctgccttgcacttattcaaaacaacagtgaattctttgatttcagatcaactactgatgaggaaccacttgagagatctgatgggggtgccatattgcaattactcaaagttttggtacctagaacatgcaaagaccggcgaaactagtgtccccaagtgctggcttgtcaccaatggttcttacttaaatgagacccacttcagtgatcaaatcgaacaggaagccgataacatgattacagagatgttgaggaaggattacataaagaggcaggggagtacccccctagcattgatggaccttctgatgttttccacatctgcatatctagtcagcatcttcctgcaccttgtcaaaataccaacacacaggcacataaaaggtggctcatgtccaaagccacaccgattaaccaacaaaggaatttgtagttgtggtgcatttaaggtgcctggtgtaaaaaccgtctggaaaagacgctgaagaacagcgcctccctgactctccacctcgaaagaggtggagagtcagggaggcccagagggtcttagagtgtcacaacatttgggcctctaaaaattaggtcatgtggcagaatgttgtgaacagttttcagatctgggagccttgctttggaggcgctttcaaaaatgatgcagtccatgagtgcacagtgcggggtgatctctttcttctttttgtcccttactattccagtatgcatcttacacaaccagccatatttgtcccacactttgtcttcatactccctcgaagcttccctggtcatttcaacatcgataagcttaatgtccttcctattctgtgagtccagaagctttctgatgtcatcggagccttgacagcttagaaccatcccctgcggaagagcacctataactgacgaggtcaacccgggttgcgcattgaagaggtcggcaagatccatgccgtgtgagtacttggaatcttgcttgaattgtttttgatcaacgggttccctgtaaaagtgtatgaactgcccgttctgtggttggaaaattgctatttccactggatcattaaatctaccctcaatgtcaatccatgtaggagcgttggggtcaattcctcccatgaggtcttttaaaagcattgtctggctgtagcttaagcccacctgaggtggacctgctgctccaggcgctggcctgggtgaattgactgcaggtttctcgcttgtgagatcaattgttgtgttttcccatgctctccccacaatcgatgttctacaagctatgtatggccatccttcacctgaaaggcaaactttatagaggatgttttcataagggttcctgtccccaacttggtctgaaacaaacatgttgagttttctcttggccccgagaactgccttcaagaggtcctcgctgttgcttggcttgatcaaaattgactctaacatgttacccccatccaacagggctgcccctgccttcacggcagcaccaagactaaagttatagccagaaatgttgatgctggactgctgttcagtgatgacccccagaactgggtgcttgtctttcagcctttcaagatcattaagatttggatacttgactgtgtaaagcaagccaaggtctgtgagcgcttgtacaacgtcattgagcggagtctgtgactgtttggccatacaagccatagttagacttggcattgtgccaaattgattgttcaaaagtgatgagtctttcacatcccaaactcttaccacaccacttgcaccctgctgaggctttctcatcccaactatctgtaggatctgagatctttggtctagttgctgtgttgttaagttccccatatatacccctgaagcctggggcctttcagacctcatgatcttggccttcagcttctcaaggtcagccgcaagagacatcagttcttctgcactgagcctccccactttcaaaacattcttctttgatgttgactttaaatccacaagagaatgtacagtctggttgagacttctgagtctctgtaggtctttgtcatctctcttttccttcctcatgatcctctgaacattgctgacctcagagaagtccaacccattcagaaggttggttgcatccttaatgacagcagccttcacatctgatgtgaagctctgcaattctcttctcaatgcttgcgtccattggaagctcttaacttccttagacaaggacatcttgttgctcaatggtttctcaagacaaatgcgcaatcaaatgcctaggatccactgtgcg

SEQ ID NO: 12 - DNA, 3377 bp, synthetic construct
  source 1..3377: mol_type = other DNA; note = lymphocytic choriomeningitis virus clone 13 segment S, complete cDNA sequence (GenBank: DQ361065.2)
gcgcaccggggatcctaggctttttggattgcgctttcctctagatcaactgggtgtcaggccctatcctacagaaggatgggtcagattgtgacaatgtttgaggctctgcctcacatcatcgatgaggtgatcaacattgtcattattgtgcttatcgtgatcacgggtatcaaggctgtctacaattttgccacctgtgggatattcgcattgatcagtttcctacttctggctggcaggtcctgtggcatgtacggtcttaagggacccgacatttacaaaggagtttaccaatttaagtcagtggagtttgatatgtcacatctgaacctgaccatgcccaacgcatgttcagccaacaactcccaccattacatcagtatggggacttctggactagaattgaccttcaccaatgattccatcatcagtcacaacttttgcaatctgacctctgccttcaacaaaaagacctttgaccacacactcatgagtatagtttcgagcctacacctcagtatcagagggaactccaactataaggcagtatcctgcgacttcaacaatggcataaccatccaatacaacttgacattctcagatgcacaaagtgctcagagccagtgtagaaccttcagaggtagagtcctagatatgtttagaactgccttcggggggaaatacatgaggagtggctggggctggacaggctcagatggcaagaccacctggtgtagccagacgagttaccaatacctgattatacaaaatagaacctgggaaaaccactgcacatatgcaggtccttttgggatgtccaggattctcctttcccaagagaagactaagttcctcactaggagactagcgggcacattcacctggactttgtcagactcttcaggggtggagaatccaggtggttattgcctgaccaaatggatgattcttgctgcagagcttaagtgtttcgggaacacagcagttgcgaaatgcaatgtaaatcatgatgaagaattctgtgacatgctgcgactaattgactacaacaaggctgctttgagtaagttcaaagaggacgtagaatctgccttgcacttattcaaaacaacagtgaattctttgatttcagatcaactactgatgaggaaccacttgagagatctgatgggggtgccatattgcaattactcaaagttttggtacctagaacatgcaaagaccggcgaaactagtgtccccaagtgctggcttgtcaccaatggttcttacttaaatgagacccacttcagtgaccaaatcgaacaggaagccgataacatgattacagagatgttgaggaaggattacataaagaggcaggggagtacccccctagcattgatggaccttctgatgttttccacatctgcatatctagtcagcatcttcctgcaccttgtcaaaataccaacacacaggcacataaaaggtggctcatgtccaaagccacaccgattaaccaacaaaggaatttgtagttgtggtgcatttaaggtgcctggtgtaaaaaccgtctggaaaagacgctgaagaacagcgcctccctgactctccacctcgaaagaggtggagagtcagggaggcccagagggtcttagagtgtcacaacatttgggcctctaaaaattaggtcatgtggcagaatgttgtgaacagttttcagatctgggagccttgctttggaggcgctttcaaaaatgatgcagtccatgagtgcacagtgcggggtgatctctttcttctttttgtcccttactattccagtatgcatcttacacaaccagccatatttgtcccacactttgtcttcatactccctcgaagcttccctggtcatttcaacatcgataagcttaatgtccttcctattctgtgagtccagaagctttctgatgtcatcggagccttgacagcttagaaccatcccctgcggaagagcacctataactgacgaggtcaacccgggttgcgcattgaagaggtcggcaagatccatgccgtgtgagtacttggaatcttgcttgaattgtttttgatcaacgggttccctgtaaaagtgtatgaactgcccgttctgtggttggaaaattgctatttccactggatcattaaatctaccctcaatgtcaatccatgtaggagcgttggggtcaattcctcccatgaggtcttttaaaagcattgtctggctgtagcttaagcccacctgaggtggacctgctgctccaggcgctggcctgggtgaattgactgcaggtttctcgcttgtgagatcaattgttgtgttttcccatgctctccccacaatcgatgttctacaagctatgtatggccatccttcacctgaaaggcaaactttatagaggatgttttcataagggttcctgtccccaacttggtctgaaacaaacatgttgagttttctcttggccccgagaactgccttcaagaggtcctcgctgttgcttggcttgatcaaaattgactctaacatgttacccccatccaacagggctgcccctgccttcacggcagcaccaagactaaagttatagccagaaatgttgatgctggactgctgttcagtgatgacccccagaactgggtgcttgtctttcagcctttcaagatcattaagatttggatacttgactgtgtaaagcaagccaaggtctgtgagcgcttgtacaacgtcattgagcggagtctgtgactgtttggccatacaagccatagttagacttggcattgtgccaaattgattgttcaaaagtgatgagtctttcacatcccaaactcttaccacaccacttgcaccctgctgaggctttctcatcccaactatctgtaggatctgagatctttggtctagttgctgtgttgttaagttccccatatatacccctgaagcctggggcctttcagacctcatgatcttggccttcagcttctcaaggtcagccgcaagagacatcagttcttctgcactgagcctccccactttcaaaacattcttctttgatgttgactttaaatccacaagagaatgtacagtctggttgagacttctgagtctctgtaggtctttgtcatctctcttttccttcctcatgatcctctgaacattgctgacctcagagaagtccaacccattcagaaggttggttgcatccttaatgacagcagccttcacatctgatgtgaagctctgcaattctcttctcaatgcttgcgtccattggaagctcttaacttccttagacaaggacatcttgttgctcaatggtttctcaagacaaatgcgcaatcaaatgcctaggatccactgtgcg

SEQ ID NO: 13 - DNA, 7205 bp, synthetic construct
  source 1..7205: mol_type = other DNA; note = lymphocytic choriomeningitis strain MP segment L, complete cDNA sequence
gcgcaccggggatcctaggcatttttgttgcgcattttgttgtgttatttgttgcacagcccttcatcgtgggaccttcacaaacaaaccaaaccaccagccatgggccaaggcaagtccaaagagggaagggatgccagcaatacgagcagagctgaaattctgccagacaccacctatctcggacctctgaactgcaagtcatgctggcagagatttgacagtttagtcagatgccatgaccactatctctgcagacactgcctgaacctcctgctgtcagtctccgacaggtgccctctctgcaaacatccattgccaaccaaactgaaaatatccacggccccaagctctccacccccttacgaggagtgacgccccgagccccaacaccgacacaaggaggccaccaacacaacgcccaacacggaacacacacacacacacccacacacacatccacacacacgcgcccccacaacgggggcgcccccccgggggtggccccccgggtgctcgggcggagccccacggagaggccaattagtcgatctcctcgaccaccgacttggtcagccagtcatcacaggacttgcccttaagtctgtacttgcccacaactgtttcatacatcaccgtgttctttgacttactgaaacatagcctacagtctttgaaagtgaaccagtcaggcacaagtgacagcggtaccagtagaatggatctatctatacacaactcttggagaattgtgctaatttccgacccctgtagatgctcaccagttctgaatcgatgtagaagaaggctcccaaggacgtcatcaaaatttccataaccctcgagctctgccaagaaaactctcatatccttggtctccagtttcacaacgatgttctgaacaaggcttcttccctcaaaaagagcacccattctcacagtcaagggcacaggctcccattcaggcccaatcctctcaaaatcaagggatctgatcccgtccagtattttccttgagcctatcagctcaagctcaagagagtcaccgagtatcagggggtcctccatatagtcctcaaactcttcagacctaatgtcaaaaacaccatcgttcaccttgaagatagagtctgatctcaacaggtggaggcattcgtccaagaaccttctgtccacctcacctttaaagaggtgagagcatgataggaactcagctacacctggaccttgtaactggcacttcactaaaaagatcaatgaaaacttcctcaaacaatcagtgttattctggttgtgagtgaaatctactgtaattgagaactctagcactccctctgtattatttatcatgtaatcccacaagtttctcaaagacttgaatgcctttggatttgtcaagccttgtttgattagcatggcagcattgcacacaatatctcccaatcggtaagagaaccatccaaatccaaattgcaagtcattcctaaacatgggcctctccatatttttgttcactacttttaagatgaatgattggaaaggccccaatgcttcagcgccatcttcagatggcatcatgtctttatgagggaaccatgaaaaacttcctagagttctgcttgttgctacaaattctcgtacaaatgactcaaaatacacttgttttaaaaagtttttgcagacatcccttgtactaacgacaaattcatcaacaaggcttgagtcagagcgctgatgggaatttacaagatcagaaaatagaacagtgtagtgttcgtccctcttccacttaactacatgagaaatgagcgataaagattctgaattgatatcgatcaatacgcaaaggtcaaggaatttgattctgggactccatctcatgttttttgagctcatatcagacatgaagggaagcagctgatcttcatagattttagggtacaatcgcctcacagattggattacatggtttaaacttatcttgtcctccagtagccttgaactctcaggcttccttgctacataatcacatgggttcaagtgcttgaggcttgagcttccctcattcttccctttcacaggttcagctaagacccaaacacccaactcaaaggaattactcagtgagatgcaaatatagtcccaaaggaggggcctcaagagactgatgtggtcgcagtgagcttctggatgactttgcctgtcacaaatgtacaacattatgccatcatgtctgtggattgctgtcacatgcgcatccatagctagatcctcaagcacttttctaatgtatagattgtccctatttttatttctcacacatctacttcccaaagttttgcaaagacctataaagcctgatgagatgcaactttgaaaggctgacttattgattgcttctgacagcaacttctgtgcacctcttgtgaacttactgcagagcttgttctggagtgtcttgattaatgatgggattctttcctcttggaaagtcattactgatggataaaccactttctgcctcaagaccattcttaatgggaacaactcattcaaattcagccaatttatgtttgccaattgacttagatcctcttcgaggccaaggatgtttcccaactgaagaatggcttcctttttatccctattgaagaggtctaagaagaattcttcattgaactcaccattcttgagcttatgatgtagtctccttacaagccttctcatgaccttcgtttcactaggacacaattcttcaataagcctttggattctgtaacctctagagccatccaaccaatccttgacatcagtattagtgttaagcaaaaatgggtccaagggaaagttggcatattttaagaggtctaatgttctcttctggatgcagtttaccaatgaaactggaacaccatttgcaacagcttgatcggcaattgtatctattgtttcacagagttggtgtggctctttacacttaacgttgtgtaatgctgctgacacaaattttgttaaaagtgggacctcttccccccacacataaaatctggatttaaattctgcagcaaatcgccccaccacacttttcggactgatgaacttgttaagcaagccactcaaatgagaatgaaattccagcaatacaaggacttcctcagggtcactatcaaccagttcactcaatctcctatcaaataaggtgatctgatcatcacttgatgtgtaagattctggtctctcaccaaaaatgacaccgatacaataattaatgaatctctcactgattaagccgtaaaagtcagaggcattatgtaagattccctgtcccatgtcaatgagactgcttatatgggaaggcactattcctaattcaaaatattctcgaaagattctttcagtcacagttgtctctgaacccctaagaagtttcagctttgatttgatatatgatttcatcattgcattcacaacaggaaaagggacctcaacaagtttgtgcatgtgccaagttaataaggtgctgatatgatcctttccggaacgcacatactggtcatcacccagtttgagattttgaaggagcattaaaaacaaaaatgggcacatcattggcccccatttgctatgatccatactgtagttcaacaacccctctcgcacattgatggtcattgatagaattgcattttcaaattctttgtcattgtttaagcatgaacctgagaagaagctagaaaaagactcaaaataatcctctatcaatcttgtaaacatttttgttctcaaatccccaatataaagttctctgtttcctccaacctgctctttgtatgataacgcaaacttcaaccttccggaatcaggaccaactgaagtgtatgacgttggtgactcctctgagtaaaaacataaattctttaaagcagcactcatgcattttgtcaatgatagagccttacttagagactcagaattactttccctttcactaattctaacatcttcttctagtttgtcccagtcaaacttgaaattcagaccttgtctttgcatgtgcctgtatttccctgagtatgcatttgcattcatttgcagtagaatcattttcatacacgaaaaccaatcaccctctgaaaaaaacttcctgcagaggttttttgccatttcatccagaccacattgttctttgacagctgaagtgaaatacaatggtgacagttctgtagaagtttcaatagcctcacagataaatttcatgtcatcattggtgagacaagatgggtcaaaatcttccacaagatgaaaagaaatttctgataagatgaccttccttaaatatgccattttacctgacaatatagtctgaaggtgatgcaatccttttgtattttcaaaccccacctcattttccccttcattggtcttcttgcttctttcataccgctttattgtggagttgaccttatcttctaaattcttgaagaaacttgtctcttcttccccatcaaagcatatgtctgctgagtcaccttctagtttcccagcttctgtttctttagagccgataaccaatctagagaccaactttgaaaccttgtactcgtaatctgagtggttcaatttgtacttctgctttctcatgaagctctctgtgatctgactcacagcactaacaagcaatttgttaaaatcatactctaggagccgttccccatttaaatgtttgttaacaaccacacttttgttgctggcaaggtctaatgctgttgcacacccagagttagtcatgggatccaagctattgagcctcttctcccctttgaaaatcaaagtgccattgttgaatgaggacaccatcatgctaaaggcctccagattgacacctggggttgtgcgctgacagtcaacttctttcccagtgaacttcttcatttggtcataaaaaacacactcttcctcaggggtgattgactctttagggttaacaaagaagccaaactcacttttaggctcaaagaatttctcaaagcatttaatttgatctgtcagcctatcaggggtttcctttgtgattaaatgacacaggtatgacacattcaacatgaacttgaactttgcgctcaacagtaccttttcaccagtcccaaaaacagttttgatcaaaaatctgagcaatttgtacactactttctcagcaggtgtgatcaaatcctccttcaacttgtccatcaatgatgtggatgagaagtctgagacaatggccatcactaaatacctaatgttttgaacctgtttttgattcctctttgttgggttggtgagcatgagtaataatagggttctcaatgcaatctcaacatcatcaatgctgtccttcaagtcaggacatgatctgatccatgagatcatggtgtcaatcatgttgtgcaacacttcatctgagaagattggtaaaaagaacctttttgggtctgcataaaaagagattagatggccattgggaccttgtatagaataacaccttgaggattctccagtcttttgatacagcaggtgatattcctcagagtccaattttatcacttggcaaaatacctctttacattccaccacttgataccttacagagcccaattggttttgtcttaatctagcaactgaacttgttttcatactgtttgtcaaagctagacagacagatgacaatcttttcaaactatgcatgttccttaattgttccgtattaggctggaaatcataatcttcaaactttgtataatacattataggatgagttccggacctcatgaaattctcaaactcaataaatggtatgtggcactcatgctcaagatgttcagacagaccatagtgcccaaaactaagtcccaccactgacaagcacctttgaacttttaaaatgaactcatttatggatgttctaaacaaatcctcaagagatacctttctatacgcctttgactttctcctgttccttagaagtctgatgaactcttccttggtgctatgaaagctcaccaacctatcattcacactcccatagcaacaaccaacccagtgcttatcattttttgaccctttgagtttagactgtttgatcaacgaagagagacacaagacatccaaattcagtaactgtctccttctggtgttcaataattttaaacttttaactttgttcaacatagagaggagcctctcatactcagtgctagtctcacttcctctctcataaccatgggtatctgctgtgataaatctcatcaaaggacaggattcaactgcctccttgcttagtgctgaaatgtcatcactgtcagcaagagtctcataaagctcagagaattccttaattaaatttccggggttgattttctgaaaactcctcttgagcttcccagtttccaagtctcttctaaacctgctgtaaagggagtttatgccaagaaccacatcatcgcagttcatgtttgggttgacaccatcatggcacattttcataatttcatcattgtgaaatgatcttgcatctttcaagattttcatagagtctataccggaacgcttatcaacagtggtcttgagagattcgcaaagtctgaagtactcagattcctcaaagactttctcatcttggctagaatactctaaaagtttaaacagaaggtctctgaacttgaaattcacccactctggcataaagctgttatcataatcacaccgaccatccactattgggaccaatgtgatacccgcaatggcaaggtcttctttgatacaggctagtttattggtgtcctctataaatttcttctcaaaactagctggtgtgcttctaacgaagcactcaagaagaatgagggaattgtcaatcagtttataaccatcaggaatgatcaaaggcagtcccgggcacacaatcccagactctattagaattgcctcaacagatttatcatcatggttgtgtatgcagccgctcttgtcagcactgtctatctctatacaacgcgacaaaagtttgagtccctctatcaataccattctgggttctctttgccctaaaaagttgagcttctgccttgacaacctctcatcttgttctatgtggtttaagcacaactctctcaactccgaaatagcctcatccattgcgcatcaaaaagcctaggatcctcggtgcg

SEQ ID NO: 14 - DNA, 3359 bp, synthetic construct
  source 1..3359: mol_type = other DNA; note = lymphocytic choriomeningitis strain MP segment S, complete cDNA sequence
cgcaccggggatcctaggctttttggattgcgctttcctcagctccgtcttgtgggagaatgggtcaaattgtgacgatgtttgaggctctgcctcacatcattgatgaggtcattaacattgtcattatcgtgcttattatcatcacgagcatcaaagctgtgtacaatttcgccacctgcgggatacttgcattgatcagctttctttttctggctggcaggtcctgtggaatgtatggtcttgatgggcctgacatttacaaaggggtttaccgattcaagtcagtggagtttgacatgtcttaccttaacctgacgatgcccaatgcatgttcggcaaacaactcccatcattatataagtatggggacttctggattggagttaaccttcacaaatgactccatcatcacccacaacttttgtaatctgacttccgccctcaacaagaggacttttgaccacacacttatgagtatagtctcaagtctgcacctcagcattagaggggtccccagctacaaagcagtgtcctgtgattttaacaatggcatcactattcaatacaacctgtcattttctaatgcacagagcgctctgagtcaatgtaagaccttcagggggagagtcctggatatgttcagaactgcttttggaggaaagtacatgaggagtggctggggctggacaggttcagatggcaagactacttggtgcagccagacaaactaccaatatctgattatacaaaacaggacttgggaaaaccactgcaggtacgcaggccctttcggaatgtctagaattctcttcgctcaagaaaagacaaggtttctaactagaaggcttgcaggcacattcacttggactttatcagactcatcaggagtggagaatccaggtggttactgcttgaccaagtggatgatcctcgctgcagagctcaagtgttttgggaacacagctgttgcaaagtgcaatgtaaatcatgatgaagagttctgtgatatgctacgactgattgattacaacaaggctgctttgagtaaattcaaagaagatgtagaatccgctctacatctgttcaagacaacagtgaattctttgatttctgatcagcttttgatgagaaatcacctaagagacttgatgggagtgccatactgcaattactcgaaattctggtatctagagcatgcaaagactggtgagactagtgtccccaagtgctggcttgtcagcaatggttcttatttgaatgaaacccatttcagcgaccaaattgagcaggaagcagataatatgatcacagaaatgctgagaaaggactacataaaaaggcaagggagtacccctctagccttgatggatctattgatgttttctacatcagcatatttgatcagcatctttctgcatcttgtgaggataccaacacacagacacataaagggcggctcatgcccaaaaccacatcggttaaccagcaagggaatctgtagttgtggtgcatttaaagtaccaggtgtggaaaccacctggaaaagacgctgaacagcagcgcctccctgactcaccacctcgaaagaggtggtgagtcagggaggcccagagggtcttagagtgttacgacatttggacctctgaagattaggtcatgtggtaggatattgtggacagttttcaggtcggggagccttgccttggaggcgctttcaaagatgatacagtccatgagtgcacagtgtggggtgacctctttctttttcttgtccctcactattccagtgtgcatcttgcatagccagccatatttgtcccagactttgtcctcatattctcttgaagcttctttagtcatctcaacatcgatgagcttaatgtctcttctgttttgtgaatctaggagtttcctgatgtcatcagatccctgacaacttaggaccattccctgtggaagagcacctattactgaagatgtcagcccaggttgtgcattgaagaggtcagcaaggtccatgccatgtgagtatttggagtcctgcttgaattgtttttgatcagtgggttctctatagaaatgtatgtactgcccattctgtggctgaaatattgctatttctaccgggtcattaaatctgccctcaatgtcaatccatgtaggagcgttagggtcaatacctcccatgaggtccttcagcaacattgtttggctgtagcttaagcccacctgaggtgggcccgctgccccaggcgctggtttgggtgagttggccataggcctctcatttgtcagatcaattgttgtgttctcccatgctctccctacaactgatgttctacaagctatgtatggccacccctcccctgaaagacagactttgtagaggatgttctcgtaaggattcctgtctccaacctgatcagaaacaaacatgttgagtttcttcttggccccaagaactgctttcaggagatcctcactgttgcttggcttaattaagatggattccaacatgttacccccatctaacaaggctgcccctgctttcacagcagcaccgagactgaaattgtagccagatatgttgatgctagactgctgctcagtgatgactcccaagactgggtgcttgtctttcagcctttcaaggtcacttaggttcgggtacttgactgtgtaaagcagcccaaggtctgtgagtgcttgcacaacgtcattgagtgaggtttgtgattgtttggccatacaagccattgttaagcttggcattgtgccgaattgattgttcagaagtgatgagtccttcacatcccagaccctcaccacaccatttgcactctgctgaggtctcctcattccaaccatttgcagaatctgagatctttggtcaagctgttgtgctgttaagttccccatgtagactccagaagttagaggcctttcagacctcatgattttagccttcagtttttcaaggtcagctgcaagggacatcagttcttctgcactaagcctccctacttttagaacattcttttttgatgttgactttaggtccacaagggaatacacagtttggttgaggcttctgagtctctgtaaatctttgtcatccctcttctctttcctcatgatcctctgaacattgctcacctcagagaagtctaatccattcagaaggctggtggcatccttgatcacagcagctttcacatctgatgtgaagccttgaagctctctcctcaatgcctgggtccattgaaagcttttaacttctttggacagagacattttgtcactcagtggatttccaagtcaaatgcgcaatcaaaatgcctaggatccactgtgcg

SEQ ID NO: 15 - protein, 558 aa, synthetic construct
  source 1..558: note = NP protein of the MP strain of LCMV
MSLSKEVKSFQWTQALRRELQGFTSDVKAAVIKDATSLLNGLDFSEVSNVQRIMRKEKRDDKDLQRLRSLNQTVYSLVDLKSTSKKNVLKVGRLSAEELMSLAADLEKLKAKIMRSERPLTSGVYMGNLTAQQLDQRSQILQMVGMRRPQQSANGVVRVWDVKDSSLLNNQFGTMPSLTMACMAKQSQTSLNDVVQALTDLGLLYTVKYPNLSDLERLKDKHPVLGVITEQQSSINISGYNFSLGAAVKAGAALLDGGNMLESILIKPSNSEDLLKAVLGAKKKLNMFVSDQVGDRNPYENILYKVCLSGEGWPYIACRTSVVGRAWENTTIDLTNERPMANSPKPAPGAAGPPQVGLSYSQTMLLKDLMGGIDPNAPTWIDIEGRFNDPVEIAIFQPQNGQYIHFYREPTDQKQFKQDSKYSHGMDLADLFNAQPGLTSSVIGALPQGMVLSCQGSDDIRKLLDSQNRRDIKLIDVEMTKEASREYEDKVWDKYGWLCKMHTGIVRDKKKKEVTPHCALMDCIIFESASKARLPDLKTVHNILPHDLIFRGPNVVTL

SEQ ID NO: 16 - protein, 498 aa, synthetic construct
  source 1..498: note = GP protein of the MP strain of LCMV
MGQIVTMFEALPHIIDEVINIVIIVLIIITSIKAVYNFATCGILALISFLFLAGRSCGMYGLDGPDIYKGVYRFKSVEFDMSYLNLTMPNACSANNSHHYISMGTSGLELTFTNDSIITHNFCNLTSALNKRTFDHTLMSIVSSLHLSIRGVPSYKAVSCDFNNGITIQYNLSFSNAQSALSQCKTFRGRVLDMFRTAFGGKYMRSGWGWTGSDGKTTWCSQTNYQYLIIQNRTWENHCRYAGPFGMSRILFAQEKTRFLTRRLAGTFTWTLSDSSGVENPGGYCLTKWMILAAELKCFGNTAVAKCNVNHDEEFCDMLRLIDYNKAALSKFKEDVESALHLFKTTVNSLISDQLLMRNHLRDLMGVPYCNYSKFWYLEHAKTGETSVPKCWLVSNGSYLNETHFSDQIEQEADNMITEMLRKDYIKRQGSTPLALMDLLMFSTSAYLISIFLHLVRIPTHRHIKGGSCPKPHRLTSKGICSCGAFKVPGVETTWKRR

SEQ ID NO: 17 - protein, 2209 aa, synthetic construct
  source 1..2209: note = L protein of the MP strain of LCMV
MDEAISELRELCLNHIEQDERLSRQKLNFLGQREPRMVLIEGLKLLSRCIEIDSADKSGCIHNHDDKSVEAILIESGIVCPGLPLIIPDGYKLIDNSLILLECFVRSTPASFEKKFIEDTNKLACIKEDLAIAGITLVPIVDGRCDYDNSFMPEWVNFKFRDLLFKLLEYSSQDEKVFEESEYFRLCESLKTTVDKRSGIDSMKILKDARSFHNDEIMKMCHDGVNPNMNCDDVVLGINSLYSRFRRDLETGKLKRSFQKINPGNLIKEFSELYETLADSDDISALSKEAVESCPLMRFITADTHGYERGSETSTEYERLLSMLNKVKSLKLLNTRRRQLLNLDVLCLSSLIKQSKLKGSKNDKHWVGCCYGSVNDRLVSFHSTKEEFIRLLRNRRKSKAYRKVSLEDLFRTSINEFILKVQRCLSVVGLSFGHYGLSEHLEHECHIPFIEFENFMRSGTHPIMYYTKFEDYDFQPNTEQLRNMHSLKRLSSVCLALTNSMKTSSVARLRQNQLGSVRYQVVECKEVFCQVIKLDSEEYHLLYQKTGESSRCYSIQGPNGHLISFYADPKRFFLPIFSDEVLHNMIDTMISWIRSCPDLKDSIDDVEIALRTLLLLMLTNPTKRNQKQVQNIRYLVMAIVSDFSSTSLMDKLKEDLITPAEKVVYKLLRFLIKTVFGTGEKVLLSAKFKFMLNVSYLCHLITKETPDRLTDQIKCFEKFFEPKSEFGFFVNPKESITPEEECVFYDQMKKFTGKEVDCQRTTPGVNLEAFSMMVSSFNNGTLIFKGEKRLNSLDPMTNSGCATALDLASNKSVVVNKHLNGERLLEYDFNKLLVSAVSQITESFMRKQKYKLNHSDYEYKVSKLVSRLVIGSKETEAGKLEGDSADICFDGEEETSFFKNLEDKVNSTIKRYERSKKTNEGENEVGFENTKGLHHLQTILSGKMAYLRKVILSEISFHLVEDFDPSCLTNDDMKFICEAIETSTELSPLYFTSAVKEQCGLDEMAKNLCRKFFSEGDWFSCMKMILLQMNANAYSGKYRHMQRQGLNFKFDWDKLEEDVRISERESNSESLSKALSLTKCMSAALKNLCFYSEESPTSYTSVGPDSGRLKFALSYKEQVGGNRELYIGDLRTKMFTRLIEDYFESFSSFFSGSCLNNDKEFENAILSMTINVREGLLNYSMDHSKWGPMMCPFLFLMLLQNLKLGDDQYVRSGKDHISTLLTWHMHKLVEVPFPVVNAMMKSYIKSKLKLLRGSETTVTERIFREYFELGIVPSHISSLIDMGQGILHNASDFYGLISERFINYCIGVIFGERPESYTSSDDQITLFDRRLSELVDSDPEEVLVLLEFHSHLSGLLNKFISPKSVVGRFAAEFKSRFYVWGEEVPLLTKFVSAALHNVKCKEPHQLCETIDTIADQAVANGVPVSLVNCIQKRTLDLLKYANFPLDPFLLNTNTDVKDWLDGSRGYRIQRLIEELCPSETKVMRRLVRRLHHKLKNGEFNEEFFLDLFNRDKKEAILQLGNILGLEEDLSQLANINWLNLNELFPLRMVLRQKVVYPSVMTFQEERIPSLIKTLQNKLCSKFTRGAQKLLSEAINKSAFQSCISSGFIGLCKTLGSRCVRNKNRDNLYIRKVLEDLAMDAHVTAIHRHDGIMLYICDRQSHPEAHCDHISLLRPLLWDYICISLSNSFELGVWVLAEPVKGKNEGSSSLKHLNPCDYVARKPESSRLLEDKISLNHVIQSVRRLYPKIYEDQLLPFMSDMSSKNMRWSPRIKFLDLCVLIDINSESLSLISHVVKWKRDEHYTVLFSDLVNSHQRSDSSLVDEFVVSTRDVCKNFLKQVYFESFVREFVATSRTLGSFSWFPHKDMMPSEDGAEALGPFQSFILKVVNKNMERPMFRNDLQFGFGWFSYRLGDIVCNAAMLIKQGLTNPKAFKSLRNLWDYMINNTEGVLEFSITVDFTHNQNNTDCLRKFSLIFLVKCQLQGPGVAEFLSCSHLFKGEVDRRFLDECLHLLRSDSIFKVNDGVFDIRSEEFEDYMEDPLILGDSLELELIGSRKILDGIRSLDFERIGPEWEPVPLTVRMGALFEGRSLVQNIVVKLETKDMRVFLAELEGYGNFDDVLGSLLLHRFRTGEHLQGSEISTILQELCIDRSILLVPLSLVPDWFTFKDCRLCFSKSKNTVMYETVVGKYRLKGKSCDDWLTKSVVEEID

SEQ ID NO: 18 - protein, 90 aa, synthetic construct
  source 1..90: note = Z protein of the MP strain of LCMV
MGQGKSKEGRDASNTSRAEILPDTTYLGPLNCKSCWQRFDSLVRCHDHYLCRHCLNLLLSVSDRCPLCKHPLPTKLKISTAPSSPPPYEE

SEQ ID NO: 19 - DNA, 7115 bp, synthetic construct
  source 1..7115: mol_type = other DNA; note = Junin virus Candid No.1 L segment
gcgcaccggggatcctaggcgtaacttcatcattaaaatctcagattctgctctgagtgtgacttactgcgaagaggcagacaaatgggcaactgcaacggggcatccaagtctaaccagccagactcctcaagagccacacagccagccgcagaatttaggagggtagctcacagcagtctatatggtagatataactgtaagtgctgctggtttgctgataccaatttgataacctgtaatgatcactacctttgtttaaggtgccatcagggtatgttaaggaattcagatctctgcaatatctgctggaagcccctgcccaccacaatcacagtaccggtggagccaacagcaccaccaccataggcagactgcacagggtcagacccgaccccccggggggcccccatggggaccccccgtgggggaaccccgggggtgatgcgccattagtcaatgtctttgatctcgactttgtgcttcagtggcctgcatgtcacccctttcaatctgaactgcccttggggatctgatatcagcaggtcatttaaagatctgctgaatgccaccttgaaatttgagaattccaaccagtcaccaaatttatcaagtgaacggatcaactgctctttgtgtagatcataaacgaggacaaagtcctcttgctgaaataatattgtttgtgatgttgtttttagataaggccatagttggcttaataaggtttccacactatcaatgtcctctagtgctccaattgccttgactatgacatccccagacaactcaactctatatgttgacaacctttcattacctctgtaaaagataccctctttcaagacaagaggttctcctgggttatctggcccaatgaggtcatatgcatacttgttacttagttcagaataaaagtcaccaaagttgaacttaacatggctcagaatattgtcatcatttgtcgcagcgtagcctgcatcaataaacaagccagctaggtcaaagctctcatggcctgtgaacaatggtaggctagcgataaccagtgcaccatccaacaatgagtggcttccctcagacccagaaacacattgactcattgcatccacattcagctctaattcaggggtaccgacatcatccactcctagtgaactgacaatggtgtaactgtacaccatctttcttctaagtttaaattttgtcgaaactcgtgtgtgttctacttgaatgatcaattttagtttcacagcttcttggcaagcaacattgcgcaacacagtgtgcaggtccatcatgtcttcctgaggcaacaaggagatgttgtcaacagagacaccctcaaggaaaaccttgatattatcaaagctagaaactacataacccattgcaatgtcttcaacaaacattgctcttgatactttattattcctaactgacaaggtaaaatctgtgagttcagctagatctacttgactgtcatcttctagatctagaacttcattgaaccaaaagaaggatttgagacacgatgttgacatgactagtgggtttatcatcgaagataagacaacttgcaccatgaagttcctgcaaacttgctgtgggctgatgccaacttcccaatttgtatactctgactgtctaacatgggctgaagcgcaatcactctgtttcacaatataaacattattatctcttactttcaataagtgacttataatccctaagttttcattcatcatgtctagagccacacagacatctagaaacttgagtcttccactatccaaagatctgttcacttgaagatcattcataaagggtgccaaatgttcttcaaatagtttggggtaatttcttcgtatagaatgcaatacatggttcatgcctaattggtcttctatctgtcgtactgctttgggtttaacagcccagaagaaattcttattacataagaccagaggggcctgtggactcttaatagcagaaaacacccactcccctaactcacaggcatttgtcagcaccaaagagaagtaatcccacaaaattggtttagaaaattggttaacttctttaagtgatttttgacagtaaataactttaggctttctctcacaaattccacaaagacatggcattattcgagtaaatatgtcctttatatacagaaatccgcctttaccatccctaacacacttactccccatactcttacaaaacccaatgaagcctgaggcaacagaagactgaaatgcagatttgttgattgactctgccaagatcttcttcacgccttttgtgaaatttcttgacagcctggactgtattgtccttatcaatgttggcatctcttctttctctaacactcttcgacttgtcatgagtttggtcctcaagaccaacctcaagtccccaaagctcgctaaattgacccatctgtagtctagagtttgtctgatttcatcttcactacacccggcatattgcaggaatccggataaagcctcatcccctcccctgcttatcaagttgataaggttttcctcaaagattttgcctctcttaatgtcattgaacactttcctcgcgcagttccttataaacattgtctccttatcatcagaaaaaatagcttcaattttcctctgtagacggtaccctctagacccatcaacccagtctttgacatcttgttcttcaatagctccaaacggagtctctctgtatccagagtatctaatcaattggttgactctaatggaaatctttgacactatatgagtgctaaccccattagcaatacattgatcacaaattgtgtctatggtctctgacagttgtgttggagttttacacttaacgttgtgtagagcagcagacacaaacttggtgagtaaaggagtctcttcacccatgacaaaaaatcttgacttaaactcagcaacaaaagttcctatcacactctttgggctgataaacttgtttaatttagaagataagaattcatggaagcacaccatttccagcagttctgtcctgtcttgaaacttttcatcactaaggcaaggaatttttataaggctaacctggtcatcgctggaggtataagtgacaggtatcacatcatacaataagtcaagtgcataacacagaaattgttcagtaattagcccatataaatctgatgtgttgtgcaagattccctggcccatgtccaagacagacattatatggctggggacctggtcccttgactgcagatactggtgaaaaaactcttcaccaacactagtacagtcacaacccattaaacctaaagatctcttcaatttccctacacagtaggcttctgcaacattaattggaacttcaacgaccttatgaagatgccatttgagaatgttcattactggttcaagattcacctttgttctatctctgggattcttcaattctaatgtgtacaaaaaagaaaggaaaagtgctgggctcatagttggtccccatttggagtggtcatatgaacaggacaagtcaccattgttaacagccattttcatatcacagattgcacgttcgaattccttttctgaattcaagcatgtgtatttcattgaactacccacagcttctgagaagtcttcaactaacctggtcatcagcttagtgttgaggtctcccacatacagttctctatttgagccaacctgctccttataacttagtccaaatttcaagttccctgtatttgagctgatgcttgtgaactctgtaggagagtcgtctgaatagaaacataaattccgtagggctgcatttgtaaaataacttttgtctagcttatcagcaatggcttcagaattgctttccctggtactaagccgaacctcatcctttagtctcagaacttcactggaaaagcccaatctagatctacttctatgctcataactacccaatttctgatcataatgtccttgaattaaaagatacttgaagcattcaaagaattcatcttcttggtaggctattgttgtcaaattttttaataacaaacccaaagggcagatgtcctgcggtgcttcaagaaaataagtcaatttaaatggagatagataaacagcatcacataactctttatacacatcagacctgagcacatctggatcaaaatccttcacctcatgcattgacacctctgctttaatctctctcaacactccaaaaggggcccacaatgactcaagagactctcgctcatcaacagatggattttttgatttcaacttggtgatctcaacttttgtcccctcactattagccatcttggctagtgtcatttgtacgtcatttctaataccctcaaaggcccttacttgatcctctgttaaactctcatacatcactgataattcttcttgattggttctggttcttgaaccggtgctcacaagacctgttagattttttaatattaagtagtccatggaatcaggatcaagattatacctgccttttgttttaaacctctcagccatagtagaaacgcatgttgaaacaagtttctccttatcataaacagaaagaatatttccaagttcgtcgagcttggggattaccacacttttattgcttgacagatccagagctgtgctagtgatgttaggcctgtagggattgcttttcagttcacctgtaactttaagtcttcctctattgaagagagaaatgcagaaggacaaaatctctttacacactcctggaatttgagtatctgaggaagtcttagcctctttggaaaagaatctgtccaatcctcttatcatggtgtcctcttgttccagtgttagactcccacttagaggggggtttacaacaacacaatcaaacttgactttgggctcaataaacttctcaaaacactttatttgatctgtcaggcgatcaggtgtctctttggttaccaagtgacacagataactaacatttaatagatatttaaaccttcttgcaaagtaaagatctgcatcttccccttcacccaaaattgtctggaaaagttccacagccatcctctgaatcagcacctctgatccagacatgcagtcgacccttaactttgacatcaaatccacatgatggatttgatttgcatatgccatcaagaaatatcttagaccttgtaaaaatgtctggttccttttggaaggggaacagagtacagctaacactaacaatcttaatattggccttgtcattgtcatgagttcgtggctaaaatccaaccagctggtcatttcctcacacatttcaattaacacatcctccgaaaatataggcaggaaaaatctctttggatcacagtaaaaagagccttgttcttccaataccccattgatggatagatagatagaatagcaccttgacttctcacctgttttttggtaaaacaagagaccaaatgtattctttgtcagatgaaatctttgtacataacactctcttagtctaacattcccaaaatatctagaatactctctttcattgattaacaatcgggaggaaaatgatgtcttcatcgagttgaccaatgcaagggaaatggaggacaaaatcctaaataatttcttctgctcaccttccactaagctgctgaatggctgatgtctacagattttctcaaattccttgttaatagtatatctcatcactggtctgtcagaaacaagtgcctgagctaaaatcatcaagctatccatatcagggtgttttattagtttttccagctgtgaccagagatcttgatgagagttcttcaatgttctggaacacgcttgaacccacttggggctggtcatcaatttcttccttattagtttaatcgcctccagaatatctagaagtctgtcattgactaacattaacatttgtccaacaactattcccgcatttcttaaccttacaattgcatcatcatgcgttttgaaaagatcacaaagtaaattgagtaaaactaagtccagaaacagtaaagtgtttctcctggtgttgaaaacttttagacctttcactttgttacacacggaaagggcttgaagataacacctctctacagcatcaatagatatagaattctcatctgactggctttccatgttgacttcatctattggatgcaatgcgatagagtagactacatccatcaacttgtttgcacaaaaagggcagctgggcacatcactgtctttgtggcttcctaataagatcaagtcatttataagcttagacttttgtgaaaatttgaatttccccaactgcttgtcaaaaatctccttcttaaaccaaaaccttaactttatgagttcttctcttatgacagattctctaatgtctcctctaaccccaacaaagagggattcatttaacctctcatcataacccaaagaattctttttcaagcattcgatgttttctaatcccaagctctggttttttgtgttggacaaactatggatcaatcgctggtattcttgttcttcaatattaatctcttgcataaattttgatttctttaggatgtcgatcagcaaccaccgaactctttcaacaacccaatcagcaaggaatctattgctgtagctagatctgccatcaaccacaggaaccaacgtaatccctgcccttagtaggtcggactttaggtttaagagctttgacatgtcactcttccattttctctcaaactcatcaggattgaccctaacaaaggtttccaataggatgagtgttttccctgtgagtttgaagccatccggaatgacttttggaagggtgggacatagtatgccatagtcagacaggatcacatcaacaaacttctgatctgaattgatctgacaggcgtgtgcctcacaggactcaagctctactaaacttgacagaagtttgaacccttccaacaacagagagctggggtgatgttgagataaaaagatgtccctttggtatgctagctcctgtctttctggaaaatgctttctaataaggctttttatttcatttactgattcctccatgctcaagtgccgcctaggatcctcggtgcg

SEQ ID NO: 20 - DNA, 3411 bp, synthetic construct
  source 1..3411: mol_type = other DNA; note = Junin virus Candid No. 1 S segment
gcgcaccggggatcctaggcgattttggttacgctataattgtaactgttttctgtttggacaacatcaaaaacatccattgcacaatggggcagttcattagcttcatgcaagaaataccaacctttttgcaggaggctctgaacattgctcttgttgcagtcagtctcattgccatcattaagggtatagtgaacttgtacaaaagtggtttattccaattctttgtattcctagcgcttgcaggaagatcctgcacagaagaagctttcaaaatcggactgcacactgagttccagactgtgtccttctcaatggtgggtctcttttccaacaatccacatgacctacctttgttgtgtaccttaaacaagagccatctttacattaaggggggcaatgcttcatttcagatcagctttgatgatattgcagtattgttgccacagtatgatgttataatacaacatccagcagatatgagctggtgttccaaaagtgatgatcaaatttggttgtctcagtggttcatgaatgctgtgggacatgattggcatctagacccaccatttctgtgtaggaaccgtgcaaagacagaaggcttcatctttcaagtcaacacctccaagactggtgtcaatggaaattatgctaagaagtttaagactggcatgcatcatttatatagagaatatcctgacccttgcttgaatggcaaactgtgcttaatgaaggcacaacctaccagttggcctctccaatgtccactcgaccacgttaacacattacacttccttacaagaggtaaaaacattcaacttccaaggaggtccttgaaagcattcttctcctggtctttgacagactcatccggcaaggatacccctggaggctattgtctagaagagtggatgctcgtagcagccaaaatgaagtgttttggcaatactgctgtagcaaaatgcaatttgaatcatgactctgaattctgtgacatgttgaggctctttgattacaacaaaaatgctatcaaaaccctaaatgatgaaactaagaaacaagtaaatctgatggggcagacaatcaatgccctgatatctgacaatttattgatgaaaaacaaaattagggaactgatgagtgtcccttactgcaattacacaaaattttggtatgtcaaccacacactttcaggacaacactcattaccaaggtgctggttaataaaaaacaacagctatttgaacatctctgacttccgtaatgactggatattagaaagtgacttcttaatttctgaaatgctaagcaaagagtattcggacaggcagggtaaaactcctttgactttagttgacatctgtatttggagcacagtattcttcacagcgtcactcttccttcacttggtgggtataccctcccacagacacatcaggggcgaagcatgccctttgccacacaggttgaacagcttgggtggttgcagatgtggtaagtaccccaatctaaagaaaccaacagtttggcgtagaggacactaagacctcctgagggtccccaccagcccgggcactgcccgggctggtgtggccccccagtccgcggcctggccgcggactggggaggcactgcttacagtgcataggctgccttcgggaggaacagcaagctcggtggtaatagaggtgtaggttcctcctcatagagcttcccatctagcactgactgaaacattatgcagtctagcagagcacagtgtggttcactggaggccaacttgaagggagtatccttttccctctttttcttattgacaaccactccattgtgatatttgcataagtgaccatatttctcccagacctgttgatcaaactgcctggcttgttcagatgtgagcttaacatcaaccagtttaagatctcttcttccatggaggtcaaacaacttcctgatgtcatcggatccttgagtagtcacaaccatgtctggaggcagcaagccgatcacgtaactaagaactcctggcattgcatcttctatgtccttcattaagatgccgtgagagtgtctgctaccatttttaaaccctttctcatcatgtggttttctgaagcagtgaatgtactgcttacctgcaggttggaataatgccatctcaacagggtcagtggctggtccttcaatgtcgagccaaagggtgttggtggggtcgagtttccccactgcctctctgatgacagcttcttgtatctctgtcaagttagccaatctcaaattctgaccgtttttttccggctgtctaggaccagcaactggtttccttgtcagatcaatacttgtgttgtcccatgacctgcctgtgatttgtgatctagaaccaatataaggccaaccatcgccagaaagacaaagtttgtacaaaaggttttcataaggatttctattgcctggtttctcatcaataaacatgccttctcttcgtttaacctgaatggttgattttatgagggaagagaagttttctggggtgactctgattgtttccaacatgtttccaccatcaagaatagatgctccagcctttactgcagctgaaagactgaagttgtaaccagaaatattgatggagctttcatctttagtcacaatctgaaggcagtcatgttcctgagtcagtctgtcaaggtcacttaagtttggatacttcacagtgtatagaagcccaagtgaggttaaagcttgtatgacactgttcattgtctcacctccttgaacagtcatgcatgcaattgtcaatgcaggaacagagccaaactgattgtttagctttgaagggtctttaacatcccatatcctcaccacaccatttcccccagtcccttgctgttgaaatcccagtgttctcaatatctctgatcttttagcaagttgtgactgggacaagttacccatgtaaaccccctgagagcctgtctctgctcttcttatcttgttttttaatttctcaaggtcagacgccaactccatcagttcatccctccccagatctcccaccttgaaaactgtgtttcgttgaacactcctcatggacatgagtctgtcaacctctttattcaggtccctcaacttgttgaggtcttcttccccctttttagtctttctgagtgcccgctgcacctgtgccacttggttgaagtcgatgctgtcagcaattagcttggcgtccttcaaaacatctgacttgacagtctgagtgaattggctcaaacctctccttaaggactgagtccatctaaagcttggaacctccttggagtgtgccatgccagaagttctggtgattttgatctagaatagagttgctcagtgaaagtgttagacactatgcctaggatccactgtgcg

SEQ ID NO: 21 - protein, 558 aa, synthetic construct
  source 1..558: note = NP protein of the Clone 13 strain of LCMV (GenBank Accession No. ABC96002.1; GI:86440166)
MSLSKEVKSFQWTQALRRELQSFTSDVKAAVIKDATNLLNGLDFSEVSNVQRIMRKEKRDDKDLQRLRSLNQTVHSLVDLKSTSKKNVLKVGRLSAEELMSLAADLEKLKAKIMRSERPQASGVYMGNLTTQQLDQRSQILQIVGMRKPQQGASGVVRVWDVKDSSLLNNQFGTMPSLTMACMAKQSQTPLNDVVQALTDLGLLYTVKYPNLNDLERLKDKHPVLGVITEQQSSINISGYNFSLGAAVKAGAALLDGGNMLESILIKPSNSEDLLKAVLGAKRKLNMFVSDQVGDRNPYENILYKVCLSGEGWPYIACRTSIVGRAWENTTIDLTSEKPAVNSPRPAPGAAGPPQVGLSYSQTMLLKDLMGGIDPNAPTWIDIEGRFNDPVEIAIFQPQNGQFIHFYREPVDQKQFKQDSKYSHGMDLADLFNAQPGLTSSVIGALPQGMVLSCQGSDDIRKLLDSQNRKDIKLIDVEMTREASREYEDKVWDKYGWLCKMHTGIVRDKKKKEITPHCALMDCIIFESASKARLPDLKTVHNILPHDLIFRGPNVVTL

SEQ ID NO: 22 - protein, 498 aa, synthetic construct
  source 1..498: note = GP protein of the Clone 13 strain of LCMV (GenBank Accession No. ABC96001.2; GI:116563462)
MGQIVTMFEALPHIIDEVINIVIIVLIVITGIKAVYNFATCGIFALISFLLLAGRSCGMYGLKGPDIYKGVYQFKSVEFDMSHLNLTMPNACSANNSHHYISMGTSGLELTFTNDSIISHNFCNLTSAFNKKTFDHTLMSIVSSLHLSIRGNSNYKAVSCDFNNGITIQYNLTFSDAQSAQSQCRTFRGRVLDMFRTAFGGKYMRSGWGWTGSDGKTTWCSQTSYQYLIIQNRTWENHCTYAGPFGMSRILLSQEKTKFLTRRLAGTFTWTLSDSSGVENPGGYCLTKWMILAAELKCFGNTAVAKCNVNHDEEFCDMLRLIDYNKAALSKFKEDVESALHLFKTTVNSLISDQLLMRNHLRDLMGVPYCNYSKFWYLEHAKTGETSVPKCWLVTNGSYLNETHFSDQIEQEADNMITEMLRKDYIKRQGSTPLALMDLLMFSTSAYLVSIFLHLVKIPTHRHIKGGSCPKPHRLTNKGICSCGAFKVPGVKTVWKRR

SEQ ID NO: 23 - protein, 2210 aa, synthetic construct
  source 1..2210: note = L protein of the Clone 13 strain of LCMV (GenBank Accession No. ABC96004.1; GI:86440169)
MDEIISELRELCLNYIEQDERLSRQKLNFLGQREPRMVLIEGLKLLSRCIEIDSADKSGCTHNHDDKSVETILVESGIVCPGLPLIIPDGYKLIDNSLILLECFVRSTPASFEKKFIEDTNKLACIREDLAVAGVTLVPIVDGRCDYDNSFMPEWANFKFRDLLFKLLEYSNQNEKVFEESEYFRLCESLKTTIDKRSGMDSMKILKDARSTHNDEIMRMCHEGINPNMSCDDVVFGINSLFSRFRRDLESGKLKRNFQKVNPEGLIKEFSELYENLADSDDILTLSREAVESCPLMRFITAETHGHERGSETSTEYERLLSMLNKVKSLKLLNTRRRQLLNLDVLCLSSLIKQSKFKGLKNDKHWVGCCYSSVNDRLVSFHSTKEEFIRLLRNRKKSKVFRKVSFEELFRASISEFIAKIQKCLLVVGLSFEHYGLSEHLEQECHIPFTEFENFMKIGAHPIMYYTKFEDYNFQPSTEQLKNIQSLRRLSSVCLALTNSMKTSSVARLRQNQIGSVRYQVVECKEVFCQVIKLDSEEYHLLYQKTGESSRCYSIQGPDGHLISFYADPKRFFLPIFSDEVLYNMIDIMISWIRSCPDLKDCLTDIEVALRTLLLLMLTNPTKRNQKQVQSVRYLVMAIVSDFSSTSLMDKLREDLITPAEKVVYKLLRFLIKTIFGTGEKVLLSAKFKFMLNVSYLCHLITKETPDRLTDQIKCFEKFFEPKSQFGFFVNPKEAITPEEECVFYEQMKRFTSKEIDCQHTTPGVNLEAFSLMVSSFNNGTLIFKGEKKLNSLDPMTNSGCATALDLASNKSVVVNKHLNGERLLEYDFNKLLVSAVSQITESFVRKQKYKLSHSDYEYKVSKLVSRLVIGSKGEETGRSEDNLAEICFDGEEETSFFKSLEEKVNTTIARYRRGRRANDKGDGEKLTNTKGLHHLQLILTGKMAHLRKVILSEISFHLVEDFDPSCLTNDDMKFICEAVEGSTELSPLYFTSVIKDQCGLDEMAKNLCRKFFSENDWFSCMKMILLQMNANAYSGKYRHMQRQGLNFKFDWDKLEEDVRISERESNSESLSKALSLTQCMSAALKNLCFYSEESPTSYTSVGPDSGRLKFALSYKEQVGGNRELYIGDLRTKMFTRLIEDYFESFSSFFSGSCLNNDKEFENAILSMTINVREGFLNYSMDHSKWGPMMCPFLFLMFLQNLKLGDDQYVRSGKDHVSTLLTWHMHKLVEVPFPVVNAMMKSYVKSKLKLLRGSETTVTERIFRQYFEMGIVPSHISSLIDMGQGILHNASDFYGLLSERFINYCIGVIFGERPEAYTSSDDQITLFDRRLSDLVVSDPEEVLVLLEFQSHLSGLLNKFISPKSVAGRFAAEFKSRFYVWGEEVPLLTKFVSAALHNVKCKEPHQLCETIDTIADQAIANGVPVSLVNSIQRRTLDLLKYANFPLDPFLLNTNTDVKDWLDGSRGYRIQRLIEELCPNETKVVRKLVRKLHHKLKNGEFNEEFFLDLFNRDKKEAILQLGDLLGLEEDLNQLADVNWLNLNEMFPLRMVLRQKVVYPSVMTFQEERIPSLIKTLQNKLCSKFTRGAQKLLSEAINKSAFQSCISSGFIGLCKTLGSRCVRNKNRENLYIKKLLEDLTTDDHVTRVCNRDGITLYICDKQSHPEAHRDHICLLRPLLWDYICISLSNSFELGVWVLAEPTKGKNNSENLTLKHLNPCDYVARKPESSRLLEDKVNLNQVIQSVRRLYPKIFEDQLLPFMSDMSSKNMRWSPRIKFLDLCVLIDINSESLSLISHVVKWKRDEHYTVLFSDLANSHQRSDSSLVDEFVVSTRDVCKNFLKQVYFESFVREFVATTRTLGNFSWFPHKEMMPSEDGAEALGPFQSFVSKVVNKNVERPMFRNDLQFGFGWFSYRMGDVVCNAAMLIRQGLTNPKAFKSLKDLWDYMLNYTKGVLEFSISVDFTHNQNNTDCLRKFSLIFLVRCQLQNPGVAELLSCSHLFKGEIDRRMLDECLHLLRTDSVFKVNDGVFDIRSEEFEDYMEDPLILGDSLELELLGSKRILDGIRSIDFERVGPEWEPVPLTVKMGALFEGRNLVQNIIVKLETKDMKVFLAGLEGYEKISDVLGNLFLHRFRTGEHLLGSEISVILQELCIDRSILLIPLSLLPDWFAFKDCRLCFSKSRSTLMYETVGGRFRLKGRSCDDWLGGSVAEDID

SEQ ID NO: 24 - protein, 90 aa, synthetic construct
  source 1..90: note = Z protein of the Clone 13 strain of LCMV (GenBank Accession No. ABC96003.1; GI:86440168)
MGQGKSREEKGTNSTNRAEILPDTTYLGPLSCKSCWQKFDSLVRCHDHYLCRHCLNLLLSVSDRCPLCKYPLPTRLKISTAPSSPPPYEE

SEQ ID NO: 25 - protein, 498 aa, synthetic construct
  source 1..498: note = GP protein of the WE strain of LCMV
MGQIVTMFEALPHIIDEVINIVIIVLIIITSIKAVYNFATCGILALVSFLFLAGRSCGMYGLNGPDIYKGVYQFKSVEFDMSHLNLTMPNACSANNSHHYISMGSSGLELTFTNDSILNHNFCNLTSAFNKKTFDHTLMSIVSSLHLSIRGNSNHKAVSCDFNNGITIQYNLSFSDPQSAISQCRTFRGRVLDMFRTAFGGKYMRSGWGWAGSDGKTTWCSQTSYQYLIIQNRTWENHCRYAGPFGMSRILFAQEKTKFLTRRLAGTFTWTLSDSSGVENPGGYCLTKWMILAAELKCFGNTAVAKCNVNHDEEFCDMLRLIDYNKAALSKFKQDVESALHVFKTTVNSLISDQLLMRNHLRDLMGVPYCNYSKFWYLEHAKTGETSVPKCWLVTNGSYLNETHFSDQIEQEADNMITEMLRKDYIKRQGSTPLALMDLLMFSTSAYLISIFLHLVKIPTHRHIKGGSCPKPHRLTNKGICSCGAFKVPGVKTIWKRR

SEQ ID NO: 26 - DNA, 450 bp, synthetic construct
  source 1..450: mol_type = other DNA; note = HBV HBe antigen (GenBank Accession No. E15688.1; GI: 5710371)
atggacattgacacgtataaagaatttggagctactgtggagttactctcgtttttgccttctgacttctttccttccgtcagagatctcctagacaccgcctcagctctgtatcgagaagccttagagtctcctgagcattgctcacctcaccatactgcactcaggcaagccattctctgctggggggaattgatgactctagctacctgggtgggtaataatttggaagatccagcatccagggatctagtagtcaattatgttaatactaacatgggtttaaagatcaggcaactattgtggtttcatatatcttgccttacttttggaagagagactgtacttgaatatttggtctctttcggagtgtggattcgcactcctccagcctatagaccaccaaatgcccctatcttatcaacacttccggaaactactgttgtttaa